European Patent Application EP 4 190 820 A1, published June 7, 2023. Title: CHIMERIC ANTIGEN RECEPTOR AND USE THEREOF. Applicant: Center for Excellence in Molecular Cell Science, Chinese Academy of Sciences. The sequence listing filed with the application follows.

SEQUENCE LISTING (13 sequences)

SEQ ID NO: 1 - protein, 55 aa, Artificial Sequence
KNRKAKAKPVTRGAGAGGRQRGQNKERPPPVPNPDFEPIRKGQRDLFSGLNQRRI

SEQ ID NO: 2 - protein, 41 aa, Artificial Sequence
RSKRSRLLHSDYMNMTPRRPGPTRKHYQPYAPPRDFAAYRS

SEQ ID NO: 3 - protein, 112 aa, Artificial Sequence
RVKFSRSADAPAYQQGQNQLYNELNLGRREEYDVLDKRRGRDPEMGGKPRRKNPQEGLYNELQKDKMAEAYSEIGMKGERRRGKGHDGLYQGLSTATKDTYDALHMQALPPR

SEQ ID NO: 4 - protein, 27 aa, Artificial Sequence
FWVLVVVGGVLACYSLLVTVAFIIFWV

SEQ ID NO: 5 - protein, 522 aa, Artificial Sequence
DIQMTQTTSSLSASLGDRVTISCRASQDISKYLNWYQQKPDGTVKLLIYHTSRLHSGVPSRFSGSGSGTDYSLTISNLEQEDIATYFCQQGNTLPYTFGGGTKLEITGSTSGSGKPGSGEGSTKGEVKLQESGPGLVAPSQSLSVTCTVSGVSLPDYGVSWIRQPPRKGLEWLGVIWGSETTYYNSALKSRLTIIKDNSKSQVFLKMNSLQTDDTAIYYCAKHYYYGGSYAMDYWGQGTSVTVSSAAAIEVMYPPPYLDNEKSNGTIIHVKGKHLCPSPLFPGPSKPFWVLVVVGGVLACYSLLVTVAFIIFWVKNRKAKAKPVTRGAGAGGRQRGQNKERPPPVPNPDFEPIRKGQRDLFSGLNQRRIRSKRSRLLHSDYMNMTPRRPGPTRKHYQPYAPPRDFAAYRSRVKFSRSADAPAYQQGQNQLYNELNLGRREEYDVLDKRRGRDPEMGGKPRRKNPQEGLYNELQKDKMAEAYSEIGMKGERRRGKGHDGLYQGLSTATKDTYDALHMQALPPR

SEQ ID NO: 6 - DNA, 1569 bp, Artificial Sequence
gacatccagatgacacagactacatcctccctgtctgcctctctgggagacagagtcaccatcagttgcagggcaagtcaggacattagtaaatatttaaattggtatcagcagaaaccagatggaactgttaaactcctgatctaccatacatcaagattacactcaggagtcccatcaaggttcagtggcagtgggtctggaacagattattctctcaccattagcaacctggagcaagaagatattgccacttacttttgccaacagggtaatacgcttccgtacacgttcggaggggggactaagttggaaataacaggctccacctctggatccggcaagcccggatctggcgagggatccaccaagggcgaggtgaaactgcaggagtcaggacctggcctggtggcgccctcacagagcctgtccgtcacatgcactgtctcaggggtctcattacccgactatggtgtaagctggattcgccagcctccacgaaagggtctggagtggctgggagtaatatggggtagtgaaaccacatactataattcagctctcaaatccagactgaccatcatcaaggacaactccaagagccaagttttcttaaaaatgaacagtctgcaaactgatgacacagccatttactactgtgccaaacattattactacggtggtagctatgctatggactactggggtcaaggaacctcagtcaccgtctcctcagcggccgcaattgaagttatgtatcctcctccttacctagacaatgagaagagcaatggaaccattatccatgtgaaagggaaacacctttgtccaagtcccctatttcccggaccttctaagcccttttgggtgctggtggtggttgggggagtcctggcttgctatagcttgctagtaacagtggcctttattattttctgggtgaagaatagaaaggccaaggccaagcctgtgacacgaggagcgggtgctggcggcaggcaaaggggacaaaacaaggagaggccaccacctgttcccaacccagactttgagcccatccggaaaggccagcgggacctgttttctggcctgaatcagagacgcatcaggagtaagaggagcaggctcctgcacagtgactacatgaacatgactccccgccgccccgggcccacccgcaagcattaccagccctatgccccaccacgcgacttcgcagcctatcgctccagagtgaagttcagcaggagcgcagacgcccccgcgtaccagcagggccagaaccagctctataacgagctcaatctaggacgaagagaggagtacgatgttttggacaagagacgtggccgggaccctgagatggggggaaagccgagaaggaagaaccctcaggaaggcctgtacaatgaactgcagaaagataagatggcggaggcctacagtgagattgggatgaaaggcgagcgccggaggggcaaggggcacgatggcctttaccagggtctcagtacagccaccaaggacacctacgacgcccttcacatgcaggccctgccccctcgctaa

SEQ ID NO: 7 - protein, 39 aa, Artificial Sequence
IEVMYPPPYLDNEKSNGTIIHVKGKHLCPSPLFPGPSKP

SEQ ID NO: 8 - DNA, 2442 bp, Artificial Sequence
atggtgagcaagggcgaggagctgttcaccggggtggtgcccatcctggtcgagctggacggcgacgtaaacggccacaagttcagcgtgtccggcgagggcgagggcgatgccacctacggcaagctgaccctgaagttcatctgcaccaccggcaagctgcccgtgccctggcccaccctcgtgaccaccctgacctacggcgtgcagtgcttcagccgctaccccgaccacatgaagcagcacgacttcttcaagtccgccatgcccgaaggctacgtccaggagcgcaccatcttcttcaaggacgacggcaactacaagacccgcgccgaggtgaagttcgagggcgacaccctggtgaaccgcatcgagctgaagggcatcgacttcaaggaggacggcaacatcctggggcacaagctggagtacaactacaacagccacaacgtctatatcatggccgacaagcagaagaacggcatcaaggtgaacttcaagatccgccacaacatcgaggacggcagcgtgcagctcgccgaccactaccagcagaacacccccatcggcgacggccccgtgctgctgcccgacaaccactacctgagcacccagtccgccctgagcaaagaccccaacgagaagcgcgatcacatggtcctgctggagttcgtgaccgccgccgggatcactctcggcatggacgagctgtacaagggaagcggagagggcagaggaagtctgctaacatgcggtgacgtcgaggagaatcctggacctatgcttctcctggtgacaagccttctgctctgtgagttaccacacccagcattcctcctgatcccatacccctacgacgtgcccgactacgccgacatccagatgacacagactacatcctccctgtctgcctctctgggagacagagtcaccatcagttgcagggcaagtcaggacattagtaaatatttaaattggtatcagcagaaaccagatggaactgttaaactcctgatctaccatacatcaagattacactcaggagtcccatcaaggttcagtggcagtgggtctggaacagattattctctcaccattagcaacctggagcaagaagatattgccacttacttttgccaacagggtaatacgcttccgtacacgttcggaggggggactaagttggaaataacaggctccacctctggatccggcaagcccggatctggcgagggatccaccaagggcgaggtgaaactgcaggagtcaggacctggcctggtggcgccctcacagagcctgtccgtcacatgcactgtctcaggggtctcattacccgactatggtgtaagctggattcgccagcctccacgaaagggtctggagtggctgggagtaatatggggtagtgaaaccacatactataattcagctctcaaatccagactgaccatcatcaaggacaactccaagagccaagttttcttaaaaatgaacagtctgcaaactgatgacacagccatttactactgtgccaaacattattactacggtggtagctatgctatggactactggggtcaaggaacctcagtcaccgtctcctcagcggccgcaattgaagttatgtatcctcctccttacctagacaatgagaagagcaatggaaccattatccatgtgaaagggaaacacctttgtccaagtcccctatttcccggaccttctaagcccttttgggtgctggtggtggttgggggagtcctggcttgctatagcttgctagtaacagtggcctttattattttctgggtgaagaatagaaaggccaaggccaagcctgtgacacgaggagcgggtgctggcggcaggcaaaggggacaaaacaaggagaggccaccacctgttcccaacccagactttgagcccatccggaaaggccagcgggacctgttttctggcctgaatcagagacgcatcaggagtaagaggagcaggctcctgcacagtgactacatgaacatgactccccgccgccccgggcccacccgcaagcattaccagccctatgccccaccacgcgacttcgcagcctatcgctccagagtgaagttcagcaggagcgcagacgcccccgcgtaccagcagggccagaaccagctctataacgagctcaatctaggacgaagagaggagtacgatgttttggacaagagacgtggccgggaccctgagatggggggaaagccgagaaggaagaaccctcaggaaggcctgtacaatgaactgcagaaagataagatggcggaggcctacagtgagattgggatgaaaggcgagcgccggaggggcaaggggcacgatggcctttaccagggtctcagtacagccaccaaggacacctacgacgcccttcacatgcaggccctgccccctcgctaa

SEQ ID NO: 9 - DNA, 2442 bp, Artificial Sequence
atggtgagcaagggcgaggagctgttcaccggggtggtgcccatcctggtcgagctggacggcgacgtaaacggccacaagttcagcgtgtccggcgagggcgagggcgatgccacctacggcaagctgaccctgaagttcatctgcaccaccggcaagctgcccgtgccctggcccaccctcgtgaccaccctgacctacggcgtgcagtgcttcagccgctaccccgaccacatgaagcagcacgacttcttcaagtccgccatgcccgaaggctacgtccaggagcgcaccatcttcttcaaggacgacggcaactacaagacccgcgccgaggtgaagttcgagggcgacaccctggtgaaccgcatcgagctgaagggcatcgacttcaaggaggacggcaacatcctggggcacaagctggagtacaactacaacagccacaacgtctatatcatggccgacaagcagaagaacggcatcaaggtgaacttcaagatccgccacaacatcgaggacggcagcgtgcagctcgccgaccactaccagcagaacacccccatcggcgacggccccgtgctgctgcccgacaaccactacctgagcacccagtccgccctgagcaaagaccccaacgagaagcgcgatcacatggtcctgctggagttcgtgaccgccgccgggatcactctcggcatggacgagctgtacaagggaagcggagagggcagaggaagtctgctaacatgcggtgacgtcgaggagaatcctggacctatgcttctcctggtgacaagccttctgctctgtgagttaccacacccagcattcctcctgatcccatacccctacgacgtgcccgactacgccgacatccagatgacacagactacatcctccctgtctgcctctctgggagacagagtcaccatcagttgcagggcaagtcaggacattagtaaatatttaaattggtatcagcagaaaccagatggaactgttaaactcctgatctaccatacatcaagattacactcaggagtcccatcaaggttcagtggcagtgggtctggaacagattattctctcaccattagcaacctggagcaagaagatattgccacttacttttgccaacagggtaatacgcttccgtacacgttcggaggggggactaagttggaaataacaggctccacctctggatccggcaagcccggatctggcgagggatccaccaagggcgaggtgaaactgcaggagtcaggacctggcctggtggcgccctcacagagcctgtccgtcacatgcactgtctcaggggtctcattacccgactatggtgtaagctggattcgccagcctccacgaaagggtctggagtggctgggagtaatatggggtagtgaaaccacatactataattcagctctcaaatccagactgaccatcatcaaggacaactccaagagccaagttttcttaaaaatgaacagtctgcaaactgatgacacagccatttactactgtgccaaacattattactacggtggtagctatgctatggactactggggtcaaggaacctcagtcaccgtctcctcagcggccgcaattgaagttatgtatcctcctccttacctagacaatgagaagagcaatggaaccattatccatgtgaaagggaaacacctttgtccaagtcccctatttcccggaccttctaagcccttttgggtgctggtggtggttgggggagtcctggcttgctatagcttgctagtaacagtggcctttattattttctgggtgaagaatagaaaggccaaggccaagcctgtgacacgaggagcgggtgctggcggcaggcaaaggggacaaaacaaggagaggccaccacctgttcccaacccagactatgagcccatccggaaaggccagcgggacctgtattctggcctgaatcagagacgcatcaggagtaagaggagcaggctcctgcacagtgactacatgaacatgactccccgccgccccgggcccacccgcaagcattaccagccctatgccccaccacgcgacttcgcagcctatcgctccagagtgaagttcagcaggagcgcagacgcccccgcgtaccagcagggccagaaccagctctataacgagctcaatctaggacgaagagaggagtacgatgttttggacaagagacgtggccgggaccctgagatggggggaaagccgagaaggaagaaccctcaggaaggcctgtacaatgaactgcagaaagataagatggcggaggcctacagtgagattgggatgaaaggcgagcgccggaggggcaaggggcacgatggcctttaccagggtctcagtacagccaccaaggacacctacgacgcccttcacatgcaggccctgccccctcgctaa

SEQ ID NO: 10 - protein, 8 aa, Artificial Sequence
KNRKAKAK

SEQ ID NO: 11 - protein, 475 aa, Artificial Sequence
DIQMTQTTSSLSASLGDRVTISCRASQDISKYLNWYQQKPDGTVKLLIYHTSRLHSGVPSRFSGSGSGTDYSLTISNLEQEDIATYFCQQGNTLPYTFGGGTKLEITGSTSGSGKPGSGEGSTKGEVKLQESGPGLVAPSQSLSVTCTVSGVSLPDYGVSWIRQPPRKGLEWLGVIWGSETTYYNSALKSRLTIIKDNSKSQVFLKMNSLQTDDTAIYYCAKHYYYGGSYAMDYWGQGTSVTVSSAAAIEVMYPPPYLDNEKSNGTIIHVKGKHLCPSPLFPGPSKPFWVLVVVGGVLACYSLLVTVAFIIFWVKNRKAKAKRSKRSRLLHSDYMNMTPRRPGPTRKHYQPYAPPRDFAAYRSRVKFSRSADAPAYQQGQNQLYNELNLGRREEYDVLDKRRGRDPEMGGKPRRKNPQEGLYNELQKDKMAEAYSEIGMKGERRRGKGHDGLYQGLSTATKDTYDALHMQALPPR

SEQ ID NO: 12 - DNA, 1428 bp, Artificial Sequence
gacatccagatgacacagactacatcctccctgtctgcctctctgggagacagagtcaccatcagttgcagggcaagtcaggacattagtaaatatttaaattggtatcagcagaaaccagatggaactgttaaactcctgatctaccatacatcaagattacactcaggagtcccatcaaggttcagtggcagtgggtctggaacagattattctctcaccattagcaacctggagcaagaagatattgccacttacttttgccaacagggtaatacgcttccgtacacgttcggaggggggactaagttggaaataacaggctccacctctggatccggcaagcccggatctggcgagggatccaccaagggcgaggtgaaactgcaggagtcaggacctggcctggtggcgccctcacagagcctgtccgtcacatgcactgtctcaggggtctcattacccgactatggtgtaagctggattcgccagcctccacgaaagggtctggagtggctgggagtaatatggggtagtgaaaccacatactataattcagctctcaaatccagactgaccatcatcaaggacaactccaagagccaagttttcttaaaaatgaacagtctgcaaactgatgacacagccatttactactgtgccaaacattattactacggtggtagctatgctatggactactggggtcaaggaacctcagtcaccgtctcctcagcggccgcaattgaagttatgtatcctcctccttacctagacaatgagaagagcaatggaaccattatccatgtgaaagggaaacacctttgtccaagtcccctatttcccggaccttctaagcccttttgggtgctggtggtggttgggggagtcctggcttgctatagcttgctagtaacagtggcctttattattttctgggtgaagaatagaaaggccaaggccaagaggagtaagaggagcaggctcctgcacagtgactacatgaacatgactccccgccgccccgggcccacccgcaagcattaccagccctatgccccaccacgcgacttcgcagcctatcgctccagagtgaagttcagcaggagcgcagacgcccccgcgtaccagcagggccagaaccagctctataacgagctcaatctaggacgaagagaggagtacgatgttttggacaagagacgtggccgggaccctgagatggggggaaagccgagaaggaagaaccctcaggaaggcctgtacaatgaactgcagaaagataagatggcggaggcctacagtgagattgggatgaaaggcgagcgccggaggggcaaggggcacgatggcctttaccagggtctcagtacagccaccaaggacacctacgacgcccttcacatgcaggccctgccccctcgctaa

SEQ ID NO: 13 - DNA, 2301 bp, Artificial Sequence
atggtgagcaagggcgaggagctgttcaccggggtggtgcccatcctggtcgagctggacggcgacgtaaacggccacaagttcagcgtgtccggcgagggcgagggcgatgccacctacggcaagctgaccctgaagttcatctgcaccaccggcaagctgcccgtgccctggcccaccctcgtgaccaccctgacctacggcgtgcagtgcttcagccgctaccccgaccacatgaagcagcacgacttcttcaagtccgccatgcccgaaggctacgtccaggagcgcaccatcttcttcaaggacgacggcaactacaagacccgcgccgaggtgaagttcgagggcgacaccctggtgaaccgcatcgagctgaagggcatcgacttcaaggaggacggcaacatcctggggcacaagctggagtacaactacaacagccacaacgtctatatcatggccgacaagcagaagaacggcatcaaggtgaacttcaagatccgccacaacatcgaggacggcagcgtgcagctcgccgaccactaccagcagaacacccccatcggcgacggccccgtgctgctgcccgacaaccactacctgagcacccagtccgccctgagcaaagaccccaacgagaagcgcgatcacatggtcctgctggagttcgtgaccgccgccgggatcactctcggcatggacgagctgtacaagggaagcggagagggcagaggaagtctgctaacatgcggtgacgtcgaggagaatcctggacctatgcttctcctggtgacaagccttctgctctgtgagttaccacacccagcattcctcctgatcccatacccctacgacgtgcccgactacgccgacatccagatgacacagactacatcctccctgtctgcctctctgggagacagagtcaccatcagttgcagggcaagtcaggacattagtaaatatttaaattggtatcagcagaaaccagatggaactgttaaactcctgatctaccatacatcaagattacactcaggagtcccatcaaggttcagtggcagtgggtctggaacagattattctctcaccattagcaacctggagcaagaagatattgccacttacttttgccaacagggtaatacgcttccgtacacgttcggaggggggactaagttggaaataacaggctccacctctggatccggcaagcccggatctggcgagggatccaccaagggcgaggtgaaactgcaggagtcaggacctggcctggtggcgccctcacagagcctgtccgtcacatgcactgtctcaggggtctcattacccgactatggtgtaagctggattcgccagcctccacgaaagggtctggagtggctgggagtaatatggggtagtgaaaccacatactataattcagctctcaaatccagactgaccatcatcaaggacaactccaagagccaagttttcttaaaaatgaacagtctgcaaactgatgacacagccatttactactgtgccaaacattattactacggtggtagctatgctatggactactggggtcaaggaacctcagtcaccgtctcctcagcggccgcaattgaagttatgtatcctcctccttacctagacaatgagaagagcaatggaaccattatccatgtgaaagggaaacacctttgtccaagtcccctatttcccggaccttctaagcccttttgggtgctggtggtggttgggggagtcctggcttgctatagcttgctagtaacagtggcctttattattttctgggtgaagaatagaaaggccaaggccaagaggagtaagaggagcaggctcctgcacagtgactacatgaacatgactccccgccgccccgggcccacccgcaagcattaccagccctatgccccaccacgcgacttcgcagcctatcgctccagagtgaagttcagcaggagcgcagacgcccccgcgtaccagcagggccagaaccagctctataacgagctcaatctaggacgaagagaggagtacgatgttttggacaagagacgtggccgggaccctgagatggggggaaagccgagaaggaagaaccctcaggaaggcctgtacaatgaactgcagaaagataagatggcggaggcctacagtgagattgggatgaaaggcgagcgccggaggggcaaggggcacgatggcctttaccagggtctcagtacagccaccaaggacacctacgacgcccttcacatgcaggccctgccccctcgctaa